European Patent Specification EP 3 446 723 B1, published April 12, 2023. Title: Pretreatment composition for dental therapy and Kit for dental tissue generation. Applicant: National Center for Geriatrics and Gerontology. The sequence listing filed with the application follows.

SEQUENCE LISTING (40 sequences)

SEQ ID NO: 1 - DNA, 20 bp, Artificial Sequence
  primer
ggacttcgagcaagagatgg

SEQ ID NO: 2 - DNA, 20 bp, Artificial Sequence
  primer
agcactgtgttggcgtacag

SEQ ID NO: 3 - DNA, 21 bp, Artificial Sequence
  primer
gaaggtccctcagacatcccc

SEQ ID NO: 4 - DNA, 21 bp, Artificial Sequence
  primer
ccctgtaggaccttcggtgac

SEQ ID NO: 5 - DNA, 21 bp, Artificial Sequence
  primer
ttctgtggctgctgctcatag

SEQ ID NO: 6 - DNA, 20 bp, Artificial Sequence
  primer
gctctctagtcgctgaaggg

SEQ ID NO: 7 - DNA, 22 bp, Artificial Sequence
  primer
ctgtactccctggtgttcactg

SEQ ID NO: 8 - DNA, 21 bp, Artificial Sequence
  primer
ggttgagcaggtagatgttgg

SEQ ID NO: 9 - DNA, 20 bp, Artificial Sequence
  primer
caagtcgcagatcttgagca

SEQ ID NO: 10 - DNA, 20 bp, Artificial Sequence
  primer
cacttgcttgaagtcgatgc

SEQ ID NO: 11 - DNA, 21 bp, Artificial Sequence
  primer
ttctgtggctgctgctcatag

SEQ ID NO: 12 - DNA, 20 bp, Artificial Sequence
  primer
gctctctagtcgctgaaggg

SEQ ID NO: 13 - DNA, 22 bp, Artificial Sequence
  primer
ctgtactccctggtgttcactg

SEQ ID NO: 14 - DNA, 21 bp, Artificial Sequence
  primer
ggttgagcaggtagatgttgg

SEQ ID NO: 15 - DNA, 21 bp, Artificial Sequence
  primer
gaaggtccctcagacatcccc

SEQ ID NO: 16 - DNA, 21 bp, Artificial Sequence
  primer
ccctgtaggaccttcggtgac

SEQ ID NO: 17 - DNA, 20 bp, Artificial Sequence
  primer
aggccttggaactcaaggat

SEQ ID NO: 18 - DNA, 20 bp, Artificial Sequence
  primer
ccctttttggacttcaggtg

SEQ ID NO: 19 - DNA, 20 bp, Artificial Sequence
  primer
ccaggagcccagctatgaac

SEQ ID NO: 20 - DNA, 19 bp, Artificial Sequence
  primer
cccagggagaaggcaactg

SEQ ID NO: 21 - DNA, 22 bp, Artificial Sequence
  primer
ggccctaaacagatgaagtgct

SEQ ID NO: 22 - DNA, 16 bp, Artificial Sequence
  primer
tgccgccatccagagg

SEQ ID NO: 23 - DNA, 20 bp, Artificial Sequence
  primer
ttggcagccttcctgatttc

SEQ ID NO: 24 - DNA, 16 bp, Artificial Sequence
  primer
tgccgccatccagagg

SEQ ID NO: 25 - DNA, 20 bp, Artificial Sequence
  primer
accaggccgtgatctctatg

SEQ ID NO: 26 - DNA, 19 bp, Artificial Sequence
  primer
tccctttgtccctggtctc

SEQ ID NO: 27 - DNA, 21 bp, Artificial Sequence
  primer
gaaggtccctcagacatcccc

SEQ ID NO: 28 - DNA, 21 bp, Artificial Sequence
  primer
ccctgtaggaccttcggtgac

SEQ ID NO: 29 - DNA, 20 bp, Artificial Sequence
  primer
aaacatccgaggacaaggtg

SEQ ID NO: 30 - DNA, 20 bp, Artificial Sequence
  primer
cgtgtacaagtctgcgtcct

SEQ ID NO: 31 - DNA, 20 bp, Artificial Sequence
  primer
atacaggcggaaccacactc

SEQ ID NO: 32 - DNA, 19 bp, Artificial Sequence
  primer
gcctggggtccacagtaat

SEQ ID NO: 33 - DNA, 20 bp, Artificial Sequence
  primer
gccccagtcacctgctgtta

SEQ ID NO: 34 - DNA, 20 bp, Artificial Sequence
  primer
tccaggtggtccatggaatc

SEQ ID NO: 35 - DNA, 20 bp, Artificial Sequence
  primer
tggtggtgatgggcgtatct

SEQ ID NO: 36 - DNA, 20 bp, Artificial Sequence
  primer
ctggccatcactgctcaaag

SEQ ID NO: 37 - DNA, 20 bp, Artificial Sequence
  primer
cctcaggaagcttgaacctg

SEQ ID NO: 38 - DNA, 20 bp, Artificial Sequence
  primer
gggaaacctagggtgtggat

SEQ ID NO: 39 - DNA, 19 bp, Artificial Sequence
  primer
gacggaaagatgtggtgtg

SEQ ID NO: 40 - DNA, 22 bp, Artificial Sequence
  primer
agacggaagttcttggtgtagg